European Patent Application EP 4 506 359 A1, published February 12, 2025. Title: TCR Targeting Cytomegalovirus Antigen, T Cell Expressing TCR, And Application. Applicant: SHANGHAI GENERAL HOSPITAL. Application WO. The sequence listing filed with the application follows.

SEQUENCE LISTING (22 sequences)

SEQ ID NO: 1 - protein, 600 aa, Homo sapiens
MGPQLLGYVVLCLLGAGPLEAQVTQNPRYLITVTGKKLTVTCSQNMNHEYMSWYRQDPGLGLRQIYYSMNVEVTDKGDVPEGYKVSRKEKRNFPLILESPSPNQTSLYFCASSLEGYTEAFFGQGTRLTVVEDLRNVTPPKVSLFEPSKAEIANKQKATLVCLARGFFPDHVELSWWVNGKEVHSGVCTDPQAYKESNYSYCLSSRLRVSATFWHNPRNHFRCQVQFHGLSEEDKWPEGSPKPVTQNISAEAWGRADCGITSASYQQGVLSATILYEILLGKATLYAVLVSTLVVMAMVKRKNSRAKRGSGATNFSLLKQAGDVEENPGPMEKNPLAAPLLILWFHLDCVSSILNVEQSPQSLHVQEGDSTNFTCSFSSSNFYALHWYRWETAKSPEALFVMTLNGDEKKKGRISATLNTKEGYSYLYIKGSQPEDSATYLCAFPYNNNDMRFGAGTRLTVEPDIQNPEPAVYQLKDPRSQDSTLCLFTDFDSQINVPKTMESGTFITDKCVLDMKAMDSKSNGAIAWSNQTSFTCQDIFKETNATYPSSDVPCDATLTEKSFETDMNLNFQNLSVMGLRILLLKVAGFNLLMTLRLWSS

SEQ ID NO: 2 - DNA, 1800 bp, Homo sapiens
  source 1..1800: mol_type = other DNA
atggggccccagcttttgggttatgtagttctttgtctcctgggcgctggaccgctggaagcacaagtcactcaaaaccctaggtacctgatcaccgtgaccggaaagaagctgactgtgacctgctctcagaacatgaaccatgaatacatgtcatggtacaggcaggatcctgggctcggacttagacagatttactactctatgaatgtggaggtgacagataaaggggatgtgccagaaggctataaggtctccaggaaggagaagagaaactttcccttgatcttggagtctccgtccccaaaccagacctctctgtacttctgcgcttcctccctcgaggggtacaccgaggcattttttggacaggggactagactgaccgtggtggaggatctgagaaatgtgactccacccaaggtctccttgtttgagccatcaaaagcagagattgcaaacaaacaaaaggctaccctcgtgtgcttggccaggggcttcttccctgaccacgtggagctgagctggtgggtgaatggcaaggaggtccacagtggggtctgcacggaccctcaggcctacaaggagagcaattatagctactgcctgagcagccgcctgagggtctctgctaccttctggcacaatcctcgcaaccacttccgctgccaagtgcagttccatgggctttcagaggaggacaagtggccagagggctcacccaaacctgtcacacagaacatcagtgcagaggcctggggccgagcagactgtgggattacctcagcatcctatcaacaaggggtcttgtctgccaccatcctctatgagatcctgctagggaaagccaccctgtatgctgtgcttgtcagtacactggtggtgatggctatggtcaaaagaaagaattcaagagccaaaagaggttctggcgccaccaacttcagcctgctgaagcaggccggcgacgtggaggagaaccccggccccatggaaaagaaccctctggctgcccccctgttgatactgtggttccacctggactgcgtgagcagcattctgaacgtcgaacagtcccctcagtctctgcacgtccaagagggagattccaccaattttacttgtagttttagctccagcaatttctacgccctgcactggtaccggtgggagaccgccaagtctcccgaagccctctttgtgatgaccctcaacggcgatgaaaaaaaaaaagggagaattagcgccaccctgaacactaaagagggctattcttacttgtatataaaagggtctcagcctgaggacagcgctacatacttgtgtgcttttccttataacaacaacgatatgaggttcggggccggaacaaggttgaccgttgagcctgacatccagaacccagaacctgctgtgtaccagttaaaagatcctcggtctcaggacagcaccctctgcctgttcaccgactttgactcccaaatcaatgtgccgaaaaccatggaatctggaacgttcatcactgacaaatgcgtgctggacatgaaagctatggattccaagagcaatggggccattgcctggagcaaccagacaagcttcacctgccaagatatcttcaaagagaccaacgccacctaccccagttcagacgttccctgtgatgccacgttgaccgagaaaagctttgaaacagatatgaacctaaactttcaaaacctgtcagttatgggactccgaatcctcctgctgaaagtagcgggatttaacctgctcatgacgctgaggctgtggtccagt

SEQ ID NO: 3 - protein, 270 aa, Homo sapiens
MEKNPLAAPLLILWFHLDCVSSILNVEQSPQSLHVQEGDSTNFTCSFSSSNFYALHWYRWETAKSPEALFVMTLNGDEKKKGRISATLNTKEGYSYLYIKGSQPEDSATYLCAFPYNNNDMRFGAGTRLTVEPDIQNPEPAVYQLKDPRSQDSTLCLFTDFDSQINVPKTMESGTFITDKCVLDMKAMDSKSNGAIAWSNQTSFTCQDIFKETNATYPSSDVPCDATLTEKSFETDMNLNFQNLSVMGLRILLLKVAGFNLLMTLRLWSS

SEQ ID NO: 4 - DNA, 810 bp, Homo sapiens
  source 1..810: mol_type = other DNA
atggaaaagaaccctctggctgcccccctgttgatactgtggttccacctggactgcgtgagcagcattctgaacgtcgaacagtcccctcagtctctgcacgtccaagagggagattccaccaattttacttgtagttttagctccagcaatttctacgccctgcactggtaccggtgggagaccgccaagtctcccgaagccctctttgtgatgaccctcaacggcgatgaaaaaaaaaaagggagaattagcgccaccctgaacactaaagagggctattcttacttgtatataaaagggtctcagcctgaggacagcgctacatacttgtgtgcttttccttataacaacaacgatatgaggttcggggccggaacaaggttgaccgttgagcctgacatccagaacccagaacctgctgtgtaccagttaaaagatcctcggtctcaggacagcaccctctgcctgttcaccgactttgactcccaaatcaatgtgccgaaaaccatggaatctggaacgttcatcactgacaaatgcgtgctggacatgaaagctatggattccaagagcaatggggccattgcctggagcaaccagacaagcttcacctgccaagatatcttcaaagagaccaacgccacctaccccagttcagacgttccctgtgatgccacgttgaccgagaaaagctttgaaacagatatgaacctaaactttcaaaacctgtcagttatgggactccgaatcctcctgctgaaagtagcgggatttaacctgctcatgacgctgaggctgtggtccagt

SEQ ID NO: 5 - protein, 304 aa, Homo sapiens
MGPQLLGYVVLCLLGAGPLEAQVTQNPRYLITVTGKKLTVTCSQNMNHEYMSWYRQDPGLGLRQIYYSMNVEVTDKGDVPEGYKVSRKEKRNFPLILESPSPNQTSLYFCASSLEGYTEAFFGQGTRLTVVEDLRNVTPPKVSLFEPSKAEIANKQKATLVCLARGFFPDHVELSWWVNGKEVHSGVCTDPQAYKESNYSYCLSSRLRVSATFWHNPRNHFRCQVQFHGLSEEDKWPEGSPKPVTQNISAEAWGRADCGITSASYQQGVLSATILYEILLGKATLYAVLVSTLVVMAMVKRKNS

SEQ ID NO: 6 - DNA, 912 bp, Homo sapiens
  source 1..912: mol_type = other DNA
atggggccccagcttttgggttatgtagttctttgtctcctgggcgctggaccgctggaagcacaagtcactcaaaaccctaggtacctgatcaccgtgaccggaaagaagctgactgtgacctgctctcagaacatgaaccatgaatacatgtcatggtacaggcaggatcctgggctcggacttagacagatttactactctatgaatgtggaggtgacagataaaggggatgtgccagaaggctataaggtctccaggaaggagaagagaaactttcccttgatcttggagtctccgtccccaaaccagacctctctgtacttctgcgcttcctccctcgaggggtacaccgaggcattttttggacaggggactagactgaccgtggtggaggatctgagaaatgtgactccacccaaggtctccttgtttgagccatcaaaagcagagattgcaaacaaacaaaaggctaccctcgtgtgcttggccaggggcttcttccctgaccacgtggagctgagctggtgggtgaatggcaaggaggtccacagtggggtctgcacggaccctcaggcctacaaggagagcaattatagctactgcctgagcagccgcctgagggtctctgctaccttctggcacaatcctcgcaaccacttccgctgccaagtgcagttccatgggctttcagaggaggacaagtggccagagggctcacccaaacctgtcacacagaacatcagtgcagaggcctggggccgagcagactgtgggattacctcagcatcctatcaacaaggggtcttgtctgccaccatcctctatgagatcctgctagggaaagccaccctgtatgctgtgcttgtcagtacactggtggtgatggctatggtcaaaagaaagaattca

SEQ ID NO: 7 - protein, 133 aa, Homo sapiens
MEKNPLAAPLLILWFHLDCVSSILNVEQSPQSLHVQEGDSTNFTCSFSSSNFYALHWYRWETAKSPEALFVMTLNGDEKKKGRISATLNTKEGYSYLYIKGSQPEDSATYLCAFPYNNNDMRFGAGTRLTVEP

SEQ ID NO: 8 - DNA, 399 bp, Homo sapiens
  source 1..399: mol_type = other DNA
atggaaaagaaccctctggctgcccccctgttgatactgtggttccacctggactgcgtgagcagcattctgaacgtcgaacagtcccctcagtctctgcacgtccaagagggagattccaccaattttacttgtagttttagctccagcaatttctacgccctgcactggtaccggtgggagaccgccaagtctcccgaagccctctttgtgatgaccctcaacggcgatgaaaaaaaaaaagggagaattagcgccaccctgaacactaaagagggctattcttacttgtatataaaagggtctcagcctgaggacagcgctacatacttgtgtgcttttccttataacaacaacgatatgaggttcggggccggaacaaggttgaccgttgagcct

SEQ ID NO: 9 - protein, 6 aa, Homo sapiens
SSNFYA

SEQ ID NO: 10 - DNA, 18 bp, Homo sapiens
  source 1..18: mol_type = other DNA
tccagcaatttctacgcc

SEQ ID NO: 11 - protein, 7 aa, Homo sapiens
MTLNGDE

SEQ ID NO: 12 - DNA, 21 bp, Homo sapiens
  source 1..21: mol_type = other DNA
atgaccctcaacggcgatgaa

SEQ ID NO: 13 - protein, 12 aa, Homo sapiens
CAFPYNNNDMRF

SEQ ID NO: 14 - DNA, 36 bp, Homo sapiens
  source 1..36: mol_type = other DNA
tgtgcttttccttataacaacaacgatatgaggttc

SEQ ID NO: 15 - protein, 131 aa, Homo sapiens
MGPQLLGYVVLCLLGAGPLEAQVTQNPRYLITVTGKKLTVTCSQNMNHEYMSWYRQDPGLGLRQIYYSMNVEVTDKGDVPEGYKVSRKEKRNFPLILESPSPNQTSLYFCASSLEGYTEAFFGQGTRLTVV

SEQ ID NO: 16 - DNA, 393 bp, Homo sapiens
  source 1..393: mol_type = other DNA
atggggccccagcttttgggttatgtagttctttgtctcctgggcgctggaccgctggaagcacaagtcactcaaaaccctaggtacctgatcaccgtgaccggaaagaagctgactgtgacctgctctcagaacatgaaccatgaatacatgtcatggtacaggcaggatcctgggctcggacttagacagatttactactctatgaatgtggaggtgacagataaaggggatgtgccagaaggctataaggtctccaggaaggagaagagaaactttcccttgatcttggagtctccgtccccaaaccagacctctctgtacttctgcgcttcctccctcgaggggtacaccgaggcattttttggacaggggactagactgaccgtggtg

SEQ ID NO: 17 - protein, 5 aa, Homo sapiens
MNHEY

SEQ ID NO: 18 - DNA, 15 bp, Homo sapiens
  source 1..15: mol_type = other DNA
atgaaccatgaatac

SEQ ID NO: 19 - protein, 6 aa, Homo sapiens
SMNVEV

SEQ ID NO: 20 - DNA, 18 bp, Homo sapiens
  source 1..18: mol_type = other DNA
tctatgaatgtggaggtg

SEQ ID NO: 21 - protein, 13 aa, Homo sapiens
CASSLEGYTEAFF

SEQ ID NO: 22 - DNA, 39 bp, Homo sapiens
  source 1..39: mol_type = other DNA
tgcgcttcctccctcgaggggtacaccgaggcatttttt